European Patent Application EP 4 541 891 A1, published April 23, 2025. Title: Novel LRP1 -binding peptide and use thereof. Applicant: 一丸ファルコス株式会社. Application JP. The sequence listing filed with the application follows.

SEQUENCE LISTING (56 sequences)

SEQ ID NO: 1 - protein, 15 aa, synthetic construct
  SITE 10: note = Nle
  SITE 14: note = Nle
  MOD_RES 1: note = N-acetyllysine labeled with 5-FAM
KGTPCTYKYXLAEXC

SEQ ID NO: 2 - protein, 15 aa, synthetic construct
  DISULFID 5..15: note = disulfide
  MOD_RES 1: note = N-acetyl lysine labeled with 5-FAM
  SITE 10: note = Nle
  SITE 14: note = Nle
KGTPCTYKYXLAEXC

SEQ ID NO: 3 - protein, 15 aa, synthetic construct
  MOD_RES 1: note = N-acetyllysine labeled with 5-FAM
  SITE 10: note = Nle
  SITE 14: note = Nle
  CROSSLNK 5..15: note = methylene thioacetal (-S-CH2-S-)
KGTPCTYKYXLAEXC

SEQ ID NO: 4 - protein, 15 aa, synthetic construct
  CROSSLNK 5..15: note = propylene thioacetal
  MOD_RES 1: note = N-acetyllysine labeled with 5-FAM
  SITE 10: note = D-Cys
  SITE 14: note = D-Cys
KGTPCTYKYXLAEXC

SEQ ID NO: 5 - protein, 15 aa, synthetic construct
  SITE 5: note = D-Cys
  MOD_RES 1: note = N-acetyllysine labeled with 5-FAM
  SITE 10: note = Nle
  SITE 14: note = Nle
KGTPCTYKYXLAEXC

SEQ ID NO: 6 - protein, 15 aa, synthetic construct
  DISULFID 5..15: note = DISULFIDE
  SITE 5: note = D-Cys
  MOD_RES 1: note = N-acetyllysine labeled with 5-FAM
  SITE 10: note = Nle
  SITE 14: note = Nle
KGTPCTYKYXLAEXC

SEQ ID NO: 7 - protein, 15 aa, synthetic construct
  CROSSLNK 5..15: note = methylene thioactal (-S-CH2-S-)
  SITE 5: note = D-Cys
  SITE 10: note = Nle
  SITE 14: note = Nle
  MOD_RES 1: note = N-acetyllysine labeled with 5-FAM
KGTPCTYKYXLAEXC

SEQ ID NO: 8 - protein, 15 aa, synthetic construct
  CROSSLNK 5..15: note = propylene thioacetal (-S-(CH3)2-S-)
  SITE 5: note = D-Cys
  SITE 10: note = Nle
  SITE 14: note = Nle
  MOD_RES 1: note = N-acetyllysine labeled with 5-FAM
KGTPCTYKYXLAEXC

SEQ ID NO: 9 - protein, 15 aa, synthetic construct
  SITE 15: note = D-Cys
  SITE 10: note = Nle
  SITE 14: note = Nle
  MOD_RES 1: note = N-acetyllysine labeled with 5-FAM
KGTPCTYKYXLAEXC

SEQ ID NO: 10 - protein, 15 aa, synthetic construct
  DISULFID 5..15: note = DISULFIDE
  SITE 15: note = D-Cys
  MOD_RES 1: note = N-acetyllysine labeled with 5-FAM
  SITE 10: note = Nle
  SITE 14: note = Nle
KGTPCTYKYXLAEXC

SEQ ID NO: 11 - protein, 15 aa, synthetic construct
  CROSSLNK 5..15: note = methylene thioacetal (-S-CH2-S-)
  SITE 15: note = D-Cys
  MOD_RES 1: note = N-acetyllysine labeled with 5-FAM
  SITE 10: note = Nle
  SITE 14: note = Nle
KGTPCTYKYXLAEXC

SEQ ID NO: 12 - protein, 15 aa, synthetic construct
  CROSSLNK 5..15: note = propylene thioacetal (-S-(CH2)3-S-)
  SITE 15: note = D-Cys
  MOD_RES 1: note = N-acetyllysine labeled with 5-FAM
  SITE 10: note = Nle
  SITE 14: note = Nle
KGTPCTYKYXLAEXC

SEQ ID NO: 13 - protein, 15 aa, synthetic construct
  SITE 5: note = D-Cys
  SITE 15: note = D-Cys
  MOD_RES 1: note = N-acetyllysine labeled with 5-FAM
  SITE 10: note = Nle
  SITE 14: note = Nle
KGTPCTYKYXLAEXC

SEQ ID NO: 14 - protein, 15 aa, synthetic construct
  SITE 5: note = D-Cys
  SITE 15: note = D-Cys
  DISULFID 5..15: note = DISULFIDE
  MOD_RES 1: note = N-acetyllysine labeled with 5-FAM
  SITE 10: note = Nle
  SITE 14: note = Nle
KGTPCTYKYXLAEXC

SEQ ID NO: 15 - protein, 15 aa, synthetic construct
  SITE 5: note = D-Cys
  SITE 15: note = D-Cys
  CROSSLNK 5..15: note = methylene thioacetal (-S-CH2-S-)
  MOD_RES 1: note = N-acetyllysine labeled with 5-FAM
  SITE 10: note = Nle
  SITE 14: note = Nle
KGTPCTYKYXLAEXC

SEQ ID NO: 16 - protein, 15 aa, synthetic construct
  SITE 5: note = D-Cys
  SITE 15: note = D-Cys
  CROSSLNK 5..15: note = propylene thioacetal (-S-(CH2)3-S-)
  MOD_RES 1: note = N-acetyllysine labeled with 5-FAM
  SITE 10: note = Nle
  SITE 14: note = Nle
KGTPCTYKYXLAEXC

SEQ ID NO: 17 - protein, 15 aa, synthetic construct
  DISULFID 5..15: note = DISULFIDE
  MOD_RES 1: note = N-acetyllysine labeled with 5-FAM
  SITE 10: note = Nle
  SITE 14: note = Nle
KGTPCSYKYXLAEXC

SEQ ID NO: 18 - protein, 15 aa, synthetic construct
  SITE 6: note = cis-4Hyp
  MOD_RES 1: note = N-acetyllysine labeled with 5-FAM
  DISULFID 5..15: note = DISULFIDE
  SITE 10: note = Nle
  SITE 14: note = Nle
KGTPCXYKYXLAEXC

SEQ ID NO: 19 - protein, 15 aa, synthetic construct
  SITE 6: note = trans-4Hyp
  MOD_RES 1: note = N-acetyllysine labeled with 5-FAM
  DISULFID 5..15: note = DISULFIDE
  SITE 10: note = Nle
  SITE 14: note = Nle
KGTPCXYKYXLAEXC

SEQ ID NO: 20 - protein, 15 aa, synthetic construct
  MOD_RES 1: note = N-acetyllysine labeled with 5-FAM
  DISULFID 5..15: note = DISULFIDE
  SITE 10: note = Nle
  SITE 14: note = Nle
KGTPCTFKYXLAEXC

SEQ ID NO: 21 - protein, 15 aa, synthetic construct
  MOD_RES 1: note = N-acetyllysine labeled with 5-FAM
  DISULFID 5..15: note = DISULFIDE
  SITE 10: note = Nle
  SITE 14: note = Nle
KGTPCTWKYXLAEXC

SEQ ID NO: 22 - protein, 15 aa, synthetic construct
  MOD_RES 1: note = N-acetyllysine labeled with 5-FAM
  DISULFID 5..15: note = DISULFIDE
  SITE 10: note = Nle
  SITE 14: note = Nle
KGTPCTHKYXLAEXC

SEQ ID NO: 23 - protein, 15 aa, synthetic construct
  SITE 8: note = Orn
  MOD_RES 1: note = N-acetyllysine labeled with 5-FAM
  DISULFID 5..15: note = DISULFIDE
  SITE 10: note = Nle
  SITE 14: note = Nle
KGTPCTYXYXLAEXC

SEQ ID NO: 24 - protein, 15 aa, synthetic construct
  MOD_RES 1: note = N-acetyllysine labeled with 5-FAM
  DISULFID 5..15: note = DISULFIDE
  SITE 10: note = Nle
  SITE 14: note = Nle
KGTPCTYRYXLAEXC

SEQ ID NO: 25 - protein, 15 aa, synthetic construct
  MOD_RES 1: note = N-acetyllysine labeled with 5-FAM
  DISULFID 5..15: note = DISULFIDE
  SITE 9: note = Nle
  SITE 10: note = Nle
  SITE 14: note = Nle
KGTPCTYKXXLAEXC

SEQ ID NO: 26 - protein, 15 aa, synthetic construct
  MOD_RES 1: note = N-acetyllysine labeled with 5-FAM
  DISULFID 5..15: note = DISULFIDE
  SITE 14: note = Nle
KGTPCTYKRRLAEXC

SEQ ID NO: 27 - protein, 15 aa, synthetic construct
  MOD_RES 1: note = N-acetyllysine labeled with 5-FAM
  DISULFID 5..15: note = DISULFIDE
  SITE 14: note = Nle
KGTPCTYKYRLAEXC

SEQ ID NO: 28 - protein, 15 aa, synthetic construct
  MOD_RES 1: note = N-acetyllysine labeled with 5-FAM
  DISULFID 5..15: note = DISULFIDE
  SITE 10: note = Nle
  SITE 14: note = Nle
KGTPCTYKYXVAEXC

SEQ ID NO: 29 - protein, 15 aa, synthetic construct
  MOD_RES 1: note = N-acetyllysine labeled with 5-FAM
  DISULFID 5..15: note = DISULFIDE
  SITE 10: note = Nle
  SITE 14: note = Nle
KGTPCTYKYXIAEXC

SEQ ID NO: 30 - protein, 15 aa, synthetic construct
  MOD_RES 1: note = N-acetyllysine labeled with 5-FAM
  SITE 10: note = Nle
  SITE 11: note = Nle
  SITE 14: note = Nle
  DISULFID 5..15: note = DISULFIDE
KGTPCTYKYXXAEXC

SEQ ID NO: 31 - protein, 15 aa, synthetic construct
  SITE 11: note = Ahe
  MOD_RES 1: note = N-acetyllysine labeled with 5-FAM
  DISULFID 5..15: note = DISULFIDE
  SITE 10: note = Nle
  SITE 14: note = Nle
KGTPCTYKYXXAEXC

SEQ ID NO: 32 - protein, 15 aa, synthetic construct
  SITE 11: note = 2-Aminooctanoic acid
  MOD_RES 1: note = N-acetyllysine labeled with 5-FAM
  DISULFID 5..15: note = DISULFIDE
  SITE 10: note = Nle
  SITE 14: note = Nle
KGTPCTYKYXXAEXC

SEQ ID NO: 33 - protein, 15 aa, synthetic construct
  SITE 12: note = D-Alanine
  MOD_RES 1: note = N-acetyllysine labeled with 5-FAM
  DISULFID 5..15: note = DISULFIDE
  SITE 10: note = Nle
  SITE 14: note = Nle
KGTPCTYKYXLAEXC

SEQ ID NO: 34 - protein, 15 aa, synthetic construct
  SITE 12: note = Aib
  MOD_RES 1: note = N-acetyllysine labeled with 5-FAM
  DISULFID 5..15: note = DISULFIDE
  SITE 10: note = Nle
  SITE 14: note = Nle
KGTPCTYKYXLXEXC

SEQ ID NO: 35 - protein, 15 aa, synthetic construct
  MOD_RES 1: note = N-acetyllysine labeled with 5-FAM
  DISULFID 5..15: note = DISULFIDE
  SITE 10: note = Nle
  SITE 14: note = Nle
KGTPCTYKYXLADXC

SEQ ID NO: 36 - protein, 15 aa, synthetic construct
  MOD_RES 1: note = N-acetyllysine labeled with 5-FAM
  DISULFID 5..15: note = DISULFIDE
  SITE 10: note = Nle
  SITE 14: note = Nle
KGTPCTYKYXLAAXC

SEQ ID NO: 37 - protein, 15 aa, synthetic construct
  MOD_RES 1: note = N-acetyllysine labeled with 5-FAM
  DISULFID 5..15: note = DISULFIDE
  SITE 10: note = Nle
  SITE 14: note = Nle
KGTPCTYKYXLAGXC

SEQ ID NO: 38 - protein, 15 aa, synthetic construct
  MOD_RES 1: note = N-acetyllysine labeled with 5-FAM
  DISULFID 5..15: note = DISULFIDE
  SITE 10: note = Nle
KGTPCTYKYXLAEVC

SEQ ID NO: 39 - protein, 15 aa, synthetic construct
  MOD_RES 1: note = N-acetyllysine labeled with 5-FAM
  DISULFID 5..15: note = DISULFIDE
  SITE 10: note = Nle
KGTPCTYKYXLAELC

SEQ ID NO: 40 - protein, 15 aa, synthetic construct
  MOD_RES 1: note = N-acetyllysine labeled with 5-FAM
  SITE 10: note = Nle
  DISULFID 5..15: note = DISULFIDE
KGTPCTYKYXLAEIC

SEQ ID NO: 41 - protein, 15 aa, synthetic construct
  SITE 14: note = Ahe
  MOD_RES 1: note = N-acetyllysine labeled with 5-FAM
  SITE 10: note = Nle
  DISULFID 5..15: note = DISULFIDE
KGTPCTYKYXLAEXC

SEQ ID NO: 42 - protein, 15 aa, synthetic construct
  SITE 14: note = 2-Aminoactanoic acid
  MOD_RES 1: note = N-acetyllysine labeled with 5-FAM
  SITE 10: note = Nle
  DISULFID 5..15: note = DISULFIDE
KGTPCTYKYXLAEXC

SEQ ID NO: 43 - protein, 16 aa, synthetic construct
  MOD_RES 1: note = N-acetyllysine labeled with 5-FAM
  DISULFID 5..16: note = DISULFIDE
  SITE 10: note = Nle
  SITE 14: note = Nle
KGTPCTYKYXLAEXPC

SEQ ID NO: 44 - protein, 16 aa, synthetic construct
  MOD_RES 1: note = N-acetyllysine labeled with 5-FAM
  DISULFID 6..16: note = DISULFIDE
  SITE 10: note = Nle
  SITE 14: note = Nle
KGTPTCYKYXLAEXPC

SEQ ID NO: 45 - protein, 15 aa, synthetic construct
  MOD_RES 1: note = N-acetyllysine labeled with Biotin
  SITE 10: note = Nle
  SITE 14: note = Nle
KGTPCTYKYXLAEXC

SEQ ID NO: 46 - protein, 15 aa, synthetic construct
  DISULFID 5..15: note = DISULFIDE
  MOD_RES 1: note = N-acetyllysine labeled with Biotin
  SITE 10: note = Nle
  SITE 14: note = Nle
KGTPCTYKYXLAEXC

SEQ ID NO: 47 - protein, 21 aa, synthetic construct
  MOD_RES 1: note = N-acetyllysine labeled with 5-FAM
KGTFFYGGSRGKRNNFKTEEY

SEQ ID NO: 48 - protein, 22 aa, synthetic construct
  MOD_RES 1: note = N-acetyllysine labeled with 5-FAM
KGTWPKHFDKHTFYSILKLGLH

SEQ ID NO: 49 - protein, 15 aa, synthetic construct
  MOD_RES 1: note = Ac-Lys(epsilon-NH-PEG4-DBCO)
  SITE 10: note = Nle
  SITE 14: note = Nle
KGTPCTYKYXLAEXC

SEQ ID NO: 50 - protein, 15 aa, synthetic construct
  MOD_RES 1: note = Ac-Lys(epsilon-NH-PEG4-BCN)
  SITE 10: note = Nle
  SITE 14: note = Nle
KGTPCTYKYXLAEXC

SEQ ID NO: 51 - protein, 15 aa, synthetic construct
  DISULFID 5..14: note = DISULFIDE
  MOD_RES 1: note = N-acetyllysine modified with azide group
  SITE 10: note = Nle
  SITE 14: note = Nle
KGTPCTYKYXLAEXC

SEQ ID NO: 52 - protein, 15 aa, synthetic construct
  MOD_RES 1: note = N-acetyllysine modified withDBCO-PEG5
  DISULFID 5..15: note = DISULFIDE
  SITE 10: note = Nle
  SITE 14: note = Nle
KGTPCTYKYXLAEXC

SEQ ID NO: 53 - protein, 14 aa, synthetic construct
  DISULFID 4..14: note = DISULFIDE
  SITE 9: note = Nle
  SITE 13: note = Nle
GTPCTYKYXLAEXC

SEQ ID NO: 54 - protein, 14 aa, synthetic construct
  MOD_RES 1: note = N3-PEG4-glycine
  DISULFID 4..14: note = DISULFIDE
  SITE 9: note = Nle
  SITE 13: note = Nle
GTPCTYKYXLAEXC

SEQ ID NO: 55 - protein, 14 aa, synthetic construct
  DISULFID 4..14: note = DISULFIDE
  MOD_RES 1: note = DBCO-PEG5-Taz-PEG4-Glycine
  SITE 9: note = Nle
  SITE 13: note = Nle
GTPCTYKYXLAEXC

SEQ ID NO: 56 - protein, 14 aa, synthetic construct
  MOD_RES 1: note = N3-PEG4-glycine
  SITE 9: note = Nle
  SITE 13: note = Nle
GTPCTYKYXLAEXC